European Patent Application EP 4 265 271 A2, published October 25, 2023. Title: VACCINE IMMUNOGENS. Applicant: Oxford University Innovation Limited. Application GB PCT/GB2020/051146, filed May 11, 2020. The sequence listing filed with the application follows.

SEQUENCE LISTING (495 sequences)

SEQ ID NO: 1 - protein, 12 aa, Plasmodium vivax
ATVRPVANVYST

SEQ ID NO: 2 - protein, 15 aa, Plasmodium vivax
AAAAASGRSKKKKWG

SEQ ID NO: 3 - protein, 8 aa, Plasmodium vivax
AAKRPSTY

SEQ ID NO: 4 - protein, 13 aa, Plasmodium vivax
AAQKKPAAPETSA

SEQ ID NO: 5 - protein, 9 aa, Plasmodium vivax
ADKEKKQLY

SEQ ID NO: 6 - protein, 13 aa, Plasmodium vivax
AGKEKDDKKKGKD

SEQ ID NO: 7 - protein, 12 aa, Plasmodium vivax
AGKKDGAKKEVA

SEQ ID NO: 8 - protein, 12 aa, Plasmodium vivax
AIEPSLAQLAQK

SEQ ID NO: 9 - protein, 13 aa, Plasmodium vivax
AIEPSLAQLAQKY

SEQ ID NO: 10 - protein, 14 aa, Plasmodium vivax
AIEPSLAQLAQKYN

SEQ ID NO: 11 - protein, 14 aa, Plasmodium vivax
AKAVKKQKKTLKPV

SEQ ID NO: 12 - protein, 11 aa, Plasmodium vivax
AKDKKQLKKPS

SEQ ID NO: 13 - protein, 13 aa, Plasmodium vivax
AKKADAKKADAKK

SEQ ID NO: 14 - protein, 13 aa, Plasmodium vivax
AKKGEAKKGEAKK

SEQ ID NO: 15 - protein, 15 aa, Plasmodium vivax
AKSKNHTNHNQNRKA

SEQ ID NO: 16 - protein, 8 aa, Plasmodium vivax
AKVVKEVK

SEQ ID NO: 17 - protein, 12 aa, Plasmodium vivax
ALFKEKKEKPRS

SEQ ID NO: 18 - protein, 12 aa, Plasmodium vivax
ANKALLPTAGDD

SEQ ID NO: 19 - protein, 12 aa, Plasmodium vivax
APISAGIKKPHR

SEQ ID NO: 20 - protein, 13 aa, Plasmodium vivax
AQKIKKKKKLTPA

SEQ ID NO: 21 - protein, 15 aa, Plasmodium vivax
AQKIKKKKKLTPAKV

SEQ ID NO: 22 - protein, 12 aa, Plasmodium vivax
AQKKPAAPETSA

SEQ ID NO: 23 - protein, 15 aa, Plasmodium vivax
ARKKPATPKKQATPK

SEQ ID NO: 24 - protein, 12 aa, Plasmodium vivax
ASGGVLPNIHNV

SEQ ID NO: 25 - protein, 11 aa, Plasmodium vivax
ASGNDKLGKKK

SEQ ID NO: 26 - protein, 8 aa, Plasmodium vivax
ASSEAQKL

SEQ ID NO: 27 - protein, 10 aa, Plasmodium vivax
ATEAATNMNA

SEQ ID NO: 28 - protein, 12 aa, Plasmodium vivax
ATRFKKNRKKRG

SEQ ID NO: 29 - protein, 14 aa, Plasmodium vivax
AVKKQKKTLKPVTK

SEQ ID NO: 30 - protein, 9 aa, Plasmodium vivax
AVKKVGKIV

SEQ ID NO: 31 - protein, 10 aa, Plasmodium vivax
AVKKVGKIVK

SEQ ID NO: 32 - protein, 11 aa, Plasmodium vivax
AVKKVGKIVKK

SEQ ID NO: 33 - protein, 13 aa, Plasmodium vivax
AVKKVGKIVKKRT

SEQ ID NO: 34 - protein, 14 aa, Plasmodium vivax
AVKKVGKIVKKRTK

SEQ ID NO: 35 - protein, 10 aa, Plasmodium vivax
AVPSSVASHG

SEQ ID NO: 36 - protein, 10 aa, Plasmodium vivax
AVSAKNPAKK

SEQ ID NO: 37 - protein, 10 aa, Plasmodium vivax
CPTQRYNFRS

SEQ ID NO: 38 - protein, 13 aa, Plasmodium vivax
DANKALLPTAGDD

SEQ ID NO: 39 - protein, 8 aa, Plasmodium vivax
DEIERVAK

SEQ ID NO: 40 - protein, 9 aa, Plasmodium vivax
DGDHSDYNT

SEQ ID NO: 41 - protein, 12 aa, Plasmodium vivax
DGNGKKFNKKPF

SEQ ID NO: 42 - protein, 12 aa, Plasmodium vivax
DGRFNILIVVKD

SEQ ID NO: 43 - protein, 10 aa, Plasmodium vivax
DIVYSLKRQG

SEQ ID NO: 44 - protein, 8 aa, Plasmodium vivax
DKEKKQLY

SEQ ID NO: 45 - protein, 8 aa, Plasmodium vivax
DKIRYEAI

SEQ ID NO: 46 - protein, 14 aa, Plasmodium vivax
DKKDDKKVKKNILK

SEQ ID NO: 47 - protein, 10 aa, Plasmodium vivax
DKKVKKNILK

SEQ ID NO: 48 - protein, 11 aa, Plasmodium vivax
DKSYLAYKTLR

SEQ ID NO: 49 - protein, 15 aa, Plasmodium vivax
DNKKAKKVGDKRKGR

SEQ ID NO: 50 - protein, 14 aa, Plasmodium vivax
DNNEHVVQEKTVSF

SEQ ID NO: 51 - protein, 12 aa, Plasmodium vivax
DNNEHVVQEKTV

SEQ ID NO: 52 - protein, 14 aa, Plasmodium vivax
DNNEHVVQEKTVSF

SEQ ID NO: 53 - protein, 15 aa, Plasmodium vivax
DSEEKEEQGQKPEKV

SEQ ID NO: 54 - protein, 8 aa, Plasmodium vivax
DSPGGEAN

SEQ ID NO: 55 - protein, 13 aa, Plasmodium vivax
DSRANAALDEPVL

SEQ ID NO: 56 - protein, 8 aa, Plasmodium vivax
EDYSPRKV

SEQ ID NO: 57 - protein, 10 aa, Plasmodium vivax
EDYSPRKVAF

SEQ ID NO: 58 - protein, 11 aa, Plasmodium vivax
EDYSPRKVAFR

SEQ ID NO: 59 - protein, 10 aa, Plasmodium vivax
EEDGYPEEGY

SEQ ID NO: 60 - protein, 15 aa, Plasmodium vivax
EEETFEEKKSEEKKD

SEQ ID NO: 61 - protein, 15 aa, Plasmodium vivax
EETLQEESNLPVKGD

SEQ ID NO: 62 - protein, 8 aa, Plasmodium vivax
EFCFTDYE

SEQ ID NO: 63 - protein, 8 aa, Plasmodium vivax
EIKRLEEV

SEQ ID NO: 64 - protein, 12 aa, Plasmodium vivax
EKFEKIKIIDFN

SEQ ID NO: 65 - protein, 9 aa, Plasmodium vivax
EKKKKKHTQ

SEQ ID NO: 66 - protein, 8 aa, Plasmodium vivax
EKLNHAVF

SEQ ID NO: 67 - protein, 9 aa, Plasmodium vivax
EVASISEKH

SEQ ID NO: 68 - protein, 13 aa, Plasmodium vivax
EVSKIDKSYLAYK

SEQ ID NO: 69 - protein, 13 aa, Plasmodium vivax
FAKSKQVNMAKTK

SEQ ID NO: 70 - protein, 13 aa, Plasmodium vivax
FAKSKQVNMAKTK

SEQ ID NO: 71 - protein, 10 aa, Plasmodium vivax
FEGEDEDEGE

SEQ ID NO: 72 - protein, 8 aa, Plasmodium vivax
FGGQTKPV

SEQ ID NO: 73 - protein, 14 aa, Plasmodium vivax
FKKKAKTTKKIVLK

SEQ ID NO: 74 - protein, 8 aa, Plasmodium vivax
FTHCTEHC

SEQ ID NO: 75 - protein, 12 aa, Plasmodium vivax
FYKRKMDKKKRN

SEQ ID NO: 76 - protein, 10 aa, Plasmodium vivax
GADKEKKQLY

SEQ ID NO: 77 - protein, 11 aa, Plasmodium vivax
GADKKKKGAVY

SEQ ID NO: 78 - protein, 9 aa, Plasmodium vivax
GAFGKPNGV

SEQ ID NO: 79 - protein, 13 aa, Plasmodium vivax
GASCGESADQSGD

SEQ ID NO: 80 - protein, 13 aa, Plasmodium vivax
GDRVRILMYPSNI

SEQ ID NO: 81 - protein, 9 aa, Plasmodium vivax
GDTELSGRF

SEQ ID NO: 82 - protein, 10 aa, Plasmodium vivax
GDTELSGRFL

SEQ ID NO: 83 - protein, 11 aa, Plasmodium vivax
GDTELSGRFLI

SEQ ID NO: 84 - protein, 10 aa, Plasmodium vivax
GGGMFNPTKV

SEQ ID NO: 85 - protein, 9 aa, Plasmodium vivax
GILHLLHKH

SEQ ID NO: 86 - protein, 13 aa, Plasmodium vivax
GILKKKKELKLKQ

SEQ ID NO: 87 - protein, 15 aa, Plasmodium vivax
GILKYPLTSEKAMKK

SEQ ID NO: 88 - protein, 10 aa, Plasmodium vivax
GISRDGRHKL

SEQ ID NO: 89 - protein, 14 aa, Plasmodium vivax
GISRDGRHKLRLTG

SEQ ID NO: 90 - protein, 15 aa, Plasmodium vivax
GISRDGRHKLRLTGG

SEQ ID NO: 91 - protein, 10 aa, Plasmodium vivax
GKAGKGTGSF

SEQ ID NO: 92 - protein, 11 aa, Plasmodium vivax
GKAGKGTGSFG

SEQ ID NO: 93 - protein, 12 aa, Plasmodium vivax
GKAGKGTGSFGK

SEQ ID NO: 94 - protein, 13 aa, Plasmodium vivax
GKAGKGTGSFGKR

SEQ ID NO: 95 - protein, 14 aa, Plasmodium vivax
GKAGKGTGSFGKRN

SEQ ID NO: 96 - protein, 15 aa, Plasmodium vivax
GKAGKGTGSFGKRNG

SEQ ID NO: 97 - protein, 9 aa, Plasmodium vivax
GKGKNKEKL

SEQ ID NO: 98 - protein, 12 aa, Plasmodium vivax
GKGKNKEKLNHA

SEQ ID NO: 99 - protein, 13 aa, Plasmodium vivax
GKGKNKEKLNHAV

SEQ ID NO: 100 - protein, 14 aa, Plasmodium vivax
GKGKNKEKLNHAVF

SEQ ID NO: 101 - protein, 15 aa, Plasmodium vivax
GKGKNKEKLNHAVFI

SEQ ID NO: 102 - protein, 11 aa, Plasmodium vivax
GKKKGADKEKK

SEQ ID NO: 103 - protein, 14 aa, Plasmodium vivax
GKKKGADKEKKQLY

SEQ ID NO: 104 - protein, 11 aa, Plasmodium vivax
GKLLKPGKVVI

SEQ ID NO: 105 - protein, 12 aa, Plasmodium vivax
GKNKEKLNHAVF

SEQ ID NO: 106 - protein, 8 aa, Plasmodium vivax
GKVHGSLA

SEQ ID NO: 107 - protein, 9 aa, Plasmodium vivax
GKVHGSLAR

SEQ ID NO: 108 - protein, 10 aa, Plasmodium vivax
GKVHGSLARA

SEQ ID NO: 109 - protein, 11 aa, Plasmodium vivax
GKVHGSLARAG

SEQ ID NO: 110 - protein, 12 aa, Plasmodium vivax
GKVHGSLARAGK

SEQ ID NO: 111 - protein, 14 aa, Plasmodium vivax
GKVHGSLARAGKVK

SEQ ID NO: 112 - protein, 8 aa, Plasmodium vivax
GLDPKFFK

SEQ ID NO: 113 - protein, 10 aa, Plasmodium vivax
GLLRGAKKTK

SEQ ID NO: 114 - protein, 14 aa, Plasmodium vivax
GLNQKQPTKGSNIQ

SEQ ID NO: 115 - protein, 8 aa, Plasmodium vivax
GLRLKEKD

SEQ ID NO: 116 - protein, 12 aa, Plasmodium vivax
GLTVEDIRNRKA

SEQ ID NO: 117 - protein, 13 aa, Plasmodium vivax
GNAKGKKPAKKVI

SEQ ID NO: 118 - protein, 11 aa, Plasmodium vivax
GNGKKFNKKPF

SEQ ID NO: 119 - protein, 9 aa, Plasmodium vivax
GPKRATKIR

SEQ ID NO: 120 - protein, 10 aa, Plasmodium vivax
GPKRATKIRK

SEQ ID NO: 121 - protein, 8 aa, Plasmodium vivax
GPVRGISL

SEQ ID NO: 122 - protein, 15 aa, Plasmodium vivax
GQTKPVFKKKAKTTK

SEQ ID NO: 123 - protein, 14 aa, Plasmodium vivax
GRETPAKGGGHNVI

SEQ ID NO: 124 - protein, 13 aa, Plasmodium vivax
GRIGRYLKKGKYA

SEQ ID NO: 125 - protein, 14 aa, Plasmodium vivax
GRIGRYLKKGKYAK

SEQ ID NO: 126 - protein, 9 aa, Plasmodium vivax
GRKSTIKPA

SEQ ID NO: 127 - protein, 14 aa, Plasmodium vivax
GRKSTIKPATGIAV

SEQ ID NO: 128 - protein, 8 aa, Plasmodium vivax
GSAEDDLK

SEQ ID NO: 129 - protein, 8 aa, Plasmodium vivax
GSGKPSGL

SEQ ID NO: 130 - protein, 8 aa, Plasmodium vivax
GSKQVHVV

SEQ ID NO: 131 - protein, 12 aa, Plasmodium vivax
GTGRKKGPNSKL

SEQ ID NO: 132 - protein, 10 aa, Plasmodium vivax
GTPIEKLHPI

SEQ ID NO: 133 - protein, 8 aa, Plasmodium vivax
GVKKDVAK

SEQ ID NO: 134 - protein, 10 aa, Plasmodium vivax
GYPSAKKRRF

SEQ ID NO: 135 - protein, 11 aa, Plasmodium vivax
HGASRYKKSRA

SEQ ID NO: 136 - protein, 9 aa, Plasmodium vivax
HGKPKHQGV

SEQ ID NO: 137 - protein, 8 aa, Plasmodium vivax
HHKYRVKR

SEQ ID NO: 138 - protein, 15 aa, Plasmodium vivax
HLPTLKKEYRRKYAA

SEQ ID NO: 139 - protein, 9 aa, Plasmodium vivax
HLSAKSRPS

SEQ ID NO: 140 - protein, 11 aa, Plasmodium vivax
HLSAKSRPSIR

SEQ ID NO: 141 - protein, 11 aa, Plasmodium vivax
HPGHQYPNALG

SEQ ID NO: 142 - protein, 10 aa, Plasmodium vivax
HQLVENADEV

SEQ ID NO: 143 - protein, 12 aa, Plasmodium vivax
HSNMHCSPYSGC

SEQ ID NO: 144 - protein, 8 aa, Plasmodium vivax
IDEHAHLV

SEQ ID NO: 145 - protein, 14 aa, Plasmodium vivax
IEKFEKESAEMGKG

SEQ ID NO: 146 - protein, 10 aa, Plasmodium vivax
IGRFFSFLVR

SEQ ID NO: 147 - protein, 11 aa, Plasmodium vivax
IGYGSNKKTKF

SEQ ID NO: 148 - protein, 9 aa, Plasmodium vivax
IHKIKKVVR

SEQ ID NO: 149 - protein, 9 aa, Plasmodium vivax
IKKERKKGI

SEQ ID NO: 150 - protein, 8 aa, Plasmodium vivax
IKSKTHSI

SEQ ID NO: 151 - protein, 10 aa, Plasmodium vivax
ILKYPLTSEK

SEQ ID NO: 152 - protein, 15 aa, Plasmodium vivax
ISKQNFAKNKKKAAN

SEQ ID NO: 153 - protein, 8 aa, Plasmodium vivax
KAFIPCLK

SEQ ID NO: 154 - protein, 11 aa, Plasmodium vivax
KAKGAKNEMVK

SEQ ID NO: 155 - protein, 10 aa, Plasmodium vivax
KALLPTAGDD

SEQ ID NO: 156 - protein, 9 aa, Plasmodium vivax
KANGDSANK

SEQ ID NO: 157 - protein, 14 aa, Plasmodium vivax
KAPRKQLASKAARK

SEQ ID NO: 158 - protein, 12 aa, Plasmodium vivax
KDAGKKDAGKKD

SEQ ID NO: 159 - protein, 9 aa, Plasmodium vivax
KDAPPPYET

SEQ ID NO: 160 - protein, 9 aa, Plasmodium vivax
KDFAKSKQV

SEQ ID NO: 161 - protein, 12 aa, Plasmodium vivax
KDGVKKDVAKKD

SEQ ID NO: 162 - protein, 13 aa, Plasmodium vivax
KDIKKERKKGIRS

SEQ ID NO: 163 - protein, 9 aa, Plasmodium vivax
KDINTIIES

SEQ ID NO: 164 - protein, 9 aa, Plasmodium vivax
KDKAGCQNK

SEQ ID NO: 165 - protein, 12 aa, Plasmodium vivax
KDSQKKGGKKKD

SEQ ID NO: 166 - protein, 14 aa, Plasmodium vivax
KDSQKKGGKKKDKK

SEQ ID NO: 167 - protein, 12 aa, Plasmodium vivax
KDVAKKDAGKKD

SEQ ID NO: 168 - protein, 10 aa, Plasmodium vivax
KDYSDNYCEK

SEQ ID NO: 169 - protein, 11 aa, Plasmodium vivax
KEDAKGGKKKK

SEQ ID NO: 170 - protein, 12 aa, Plasmodium vivax
KEGLILKKPQKV

SEQ ID NO: 171 - protein, 12 aa, Plasmodium vivax
KEKKQLYKGKVK

SEQ ID NO: 172 - protein, 9 aa, Plasmodium vivax
KEKLNHAVF

SEQ ID NO: 173 - protein, 8 aa, Plasmodium vivax
KEPIFSNT

SEQ ID NO: 174 - protein, 9 aa, Plasmodium vivax
KEPLLGGLN

SEQ ID NO: 175 - protein, 14 aa, Plasmodium vivax
KEPLLGGLNQKQPT

SEQ ID NO: 176 - protein, 15 aa, Plasmodium vivax
KEPLLGGLNQKQPTK

SEQ ID NO: 177 - protein, 10 aa, Plasmodium vivax
KFFRRRGEAT

SEQ ID NO: 178 - protein, 9 aa, Plasmodium vivax
KGAAPKKGA

SEQ ID NO: 179 - protein, 11 aa, Plasmodium vivax
KGADKEKKQLY

SEQ ID NO: 180 - protein, 12 aa, Plasmodium vivax
KGAEQNGREPNG

SEQ ID NO: 181 - protein, 11 aa, Plasmodium vivax
KGGSGGGNIKK

SEQ ID NO: 182 - protein, 8 aa, Plasmodium vivax
KGKDTCCC

SEQ ID NO: 183 - protein, 8 aa, Plasmodium vivax
KGKKNATT

SEQ ID NO: 184 - protein, 10 aa, Plasmodium vivax
KGKKPAKKVI

SEQ ID NO: 185 - protein, 8 aa, Plasmodium vivax
KGKNKEKL

SEQ ID NO: 186 - protein, 12 aa, Plasmodium vivax
KGKNKEKLNHAV

SEQ ID NO: 187 - protein, 13 aa, Plasmodium vivax
KGKNKEKLNHAVF

SEQ ID NO: 188 - protein, 13 aa, Plasmodium vivax
KGKSSRSGRSARS

SEQ ID NO: 189 - protein, 15 aa, Plasmodium vivax
KGKVKKSLGKQVGGK

SEQ ID NO: 190 - protein, 13 aa, Plasmodium vivax
KHEKPKKLNAKLR

SEQ ID NO: 191 - protein, 14 aa, Plasmodium vivax
KHEKPKKLNAKLRK

SEQ ID NO: 192 - protein, 8 aa, Plasmodium vivax
KHIKKTKM

SEQ ID NO: 193 - protein, 10 aa, Plasmodium vivax
KIFDEIIVNA

SEQ ID NO: 194 - protein, 13 aa, Plasmodium vivax
KIRDEIKRTFCQR

SEQ ID NO: 195 - protein, 11 aa, Plasmodium vivax
KKAAPKKVAAP

SEQ ID NO: 196 - protein, 9 aa, Plasmodium vivax
KKGADKEKK

SEQ ID NO: 197 - protein, 13 aa, Plasmodium vivax
KKAAARKKPATPK

SEQ ID NO: 198 - protein, 15 aa, Plasmodium vivax
KKAAQKKPAAPETSA

SEQ ID NO: 199 - protein, 10 aa, Plasmodium vivax
KKADKKDEKK

SEQ ID NO: 200 - protein, 8 aa, Plasmodium vivax
KKAPAKPQ

SEQ ID NO: 201 - protein, 14 aa, Plasmodium vivax
KKAPNTTKPKEDTK

SEQ ID NO: 202 - protein, 13 aa, Plasmodium vivax
KKDAGKKDAGKKD

SEQ ID NO: 203 - protein, 8 aa, Plasmodium vivax
KKDDKTKK

SEQ ID NO: 204 - protein, 13 aa, Plasmodium vivax
KKDDKKVKKNILK

SEQ ID NO: 205 - protein, 14 aa, Plasmodium vivax
KKDIKKERKKGIRS

SEQ ID NO: 206 - protein, 14 aa, Plasmodium vivax
KKEKAKSEKAVIKK

SEQ ID NO: 207 - protein, 14 aa, Plasmodium vivax
KKELKLKQKQEKKN

SEQ ID NO: 208 - protein, 8 aa, Plasmodium vivax
KKGIRSNP

SEQ ID NO: 209 - protein, 8 aa, Plasmodium vivax
KKGPNSKL

SEQ ID NO: 210 - protein, 13 aa, Plasmodium vivax
KKIDKKKEQLSKK

SEQ ID NO: 211 - protein, 10 aa, Plasmodium vivax
KKIGKSKQID

SEQ ID NO: 212 - protein, 13 aa, Plasmodium vivax
KKKAKTTKKIVLK

SEQ ID NO: 213 - protein, 15 aa, Plasmodium vivax
KKKELKLKQKQEKKN

SEQ ID NO: 214 - protein, 10 aa, Plasmodium vivax
KKKGADKEKK

SEQ ID NO: 215 - protein, 13 aa, Plasmodium vivax
KKKGADKEKKQLY

SEQ ID NO: 216 - protein, 8 aa, Plasmodium vivax
KKKKGAVY

SEQ ID NO: 217 - protein, 12 aa, Plasmodium vivax
KKKKWGKGKNKE

SEQ ID NO: 218 - protein, 9 aa, Plasmodium vivax
KKKLVKRST

SEQ ID NO: 219 - protein, 10 aa, Plasmodium vivax
KKKVIKEYKK

SEQ ID NO: 220 - protein, 14 aa, Plasmodium vivax
KKKVIKEYKKVLNK

SEQ ID NO: 221 - protein, 8 aa, Plasmodium vivax
KKNLKGAK

SEQ ID NO: 222 - protein, 13 aa, Plasmodium vivax
KKNLKGAKAEEGK

SEQ ID NO: 223 - protein, 9 aa, Plasmodium vivax
KKNSLHLEK

SEQ ID NO: 224 - protein, 13 aa, Plasmodium vivax
KKPATPKKQATPK

SEQ ID NO: 225 - protein, 10 aa, Plasmodium vivax
KKSDYDKLDK

SEQ ID NO: 226 - protein, 10 aa, Plasmodium vivax
KKSTAKDAKK

SEQ ID NO: 227 - protein, 12 aa, Plasmodium vivax
KKVAAGYKKLTD

SEQ ID NO: 228 - protein, 9 aa, Plasmodium vivax
KKVKKNILK

SEQ ID NO: 229 - protein, 15 aa, Plasmodium vivax
KKVKKNILKTQKTKK

SEQ ID NO: 230 - protein, 11 aa, Plasmodium vivax
KKYKNKKFKPY

SEQ ID NO: 231 - protein, 15 aa, Plasmodium vivax
KKYKNKKFKPYNLRK

SEQ ID NO: 232 - protein, 8 aa, Plasmodium vivax
KLLLCVVL

SEQ ID NO: 233 - protein, 9 aa, Plasmodium vivax
KLMHGRDIE

SEQ ID NO: 234 - protein, 9 aa, Plasmodium vivax
KMKKSIEAK

SEQ ID NO: 235 - protein, 11 aa, Plasmodium vivax
KMKEFSDAFST

SEQ ID NO: 236 - protein, 8 aa, Plasmodium vivax
KNFKKENQ

SEQ ID NO: 237 - protein, 12 aa, Plasmodium vivax
KNGIKKPKKHKF

SEQ ID NO: 238 - protein, 14 aa, Plasmodium vivax
KNGIKKPKKHKFMS

SEQ ID NO: 239 - protein, 10 aa, Plasmodium vivax
KNIKSKNGIG

SEQ ID NO: 240 - protein, 15 aa, Plasmodium vivax
KNIKSKNGIGGIPAD

SEQ ID NO: 241 - protein, 11 aa, Plasmodium vivax
KNKEKLNHAVF

SEQ ID NO: 242 - protein, 8 aa, Plasmodium vivax
KNPKCPKV

SEQ ID NO: 243 - protein, 14 aa, Plasmodium vivax
KNQTPKVPKVSKRK

SEQ ID NO: 244 - protein, 10 aa, Plasmodium vivax
KNSLTNFAVR

SEQ ID NO: 245 - protein, 15 aa, Plasmodium vivax
KNSVKSNKKVKKMIK

SEQ ID NO: 246 - protein, 9 aa, Plasmodium vivax
KNSYSAASK

SEQ ID NO: 247 - protein, 15 aa, Plasmodium vivax
KNYGLFSDNYFTTAY

SEQ ID NO: 248 - protein, 9 aa, Plasmodium vivax
KPAAPETSA

SEQ ID NO: 249 - protein, 9 aa, Plasmodium vivax
KPAAPKKPA

SEQ ID NO: 250 - protein, 8 aa, Plasmodium vivax
KPAHVTSK

SEQ ID NO: 251 - protein, 8 aa, Plasmodium vivax
KPLIKFGT

SEQ ID NO: 252 - protein, 8 aa, Plasmodium vivax
KPNRHINL

SEQ ID NO: 253 - protein, 12 aa, Plasmodium vivax
KPQKEDAKGGKK

SEQ ID NO: 254 - protein, 8 aa, Plasmodium vivax
KPSRTTIT

SEQ ID NO: 255 - protein, 10 aa, Plasmodium vivax
KQVGGKNQQV

SEQ ID NO: 256 - protein, 15 aa, Plasmodium vivax
KRNLKKSIKKKPKSK

SEQ ID NO: 257 - protein, 9 aa, Plasmodium vivax
KSIEIDDEK

SEQ ID NO: 258 - protein, 14 aa, Plasmodium vivax
KSAGADSKSLKKLD

SEQ ID NO: 259 - protein, 8 aa, Plasmodium vivax
KSAYAISK

SEQ ID NO: 260 - protein, 8 aa, Plasmodium vivax
KSDSSKIA

SEQ ID NO: 261 - protein, 10 aa, Plasmodium vivax
KSIEAKKNNK

SEQ ID NO: 262 - protein, 9 aa, Plasmodium vivax
KSNDRSYYT

SEQ ID NO: 263 - protein, 9 aa, Plasmodium vivax
KSNGKRDPK

SEQ ID NO: 264 - protein, 12 aa, Plasmodium vivax
KSNPFRGSSHAK

SEQ ID NO: 265 - protein, 8 aa, Plasmodium vivax
KSNSISLS

SEQ ID NO: 266 - protein, 8 aa, Plasmodium vivax
KSTNILGE

SEQ ID NO: 267 - protein, 11 aa, Plasmodium vivax
KSTTTGHIIYK

SEQ ID NO: 268 - protein, 8 aa, Plasmodium vivax
KTINKTID

SEQ ID NO: 269 - protein, 14 aa, Plasmodium vivax
KTINKTIDKQKKAP

SEQ ID NO: 270 - protein, 8 aa, Plasmodium vivax
KTIYNFLI

SEQ ID NO: 271 - protein, 14 aa, Plasmodium vivax
KVDKKAPAKPQKED

SEQ ID NO: 272 - protein, 10 aa, Plasmodium vivax
KVINMKKAPN

SEQ ID NO: 273 - protein, 15 aa, Plasmodium vivax
KVPVPPTQAKKPKKN

SEQ ID NO: 274 - protein, 9 aa, Plasmodium vivax
KYFLGLARE

SEQ ID NO: 275 - protein, 12 aa, Plasmodium vivax
KYQSSTASALIA

SEQ ID NO: 276 - protein, 15 aa, Plasmodium vivax
KYRQIREGLITKENK

SEQ ID NO: 277 - protein, 15 aa, Plasmodium vivax
KYYRVKGKKKILIPV

SEQ ID NO: 278 - protein, 11 aa, Plasmodium vivax
LETEREARRLR

SEQ ID NO: 279 - protein, 14 aa, Plasmodium vivax
LETYQNMKIQKQTP

SEQ ID NO: 280 - protein, 14 aa, Plasmodium vivax
LETYQNMKIQKQTP

SEQ ID NO: 281 - protein, 14 aa, Plasmodium vivax
LETYQNMKIQKQTP

SEQ ID NO: 282 - protein, 10 aa, Plasmodium vivax
LGGLNQKQPT

SEQ ID NO: 283 - protein, 9 aa, Plasmodium vivax
LGSLVGFVF

SEQ ID NO: 284 - protein, 10 aa, Plasmodium vivax
LILRAAIKTK

SEQ ID NO: 285 - protein, 9 aa, Plasmodium vivax
LLINVFLHH

SEQ ID NO: 286 - protein, 9 aa, Plasmodium vivax
LLPKKSQLK

SEQ ID NO: 287 - protein, 11 aa, Plasmodium vivax
LLPKKSQLKSG

SEQ ID NO: 288 - protein, 11 aa, Plasmodium vivax
LNALENPPKPG

SEQ ID NO: 289 - protein, 13 aa, Plasmodium vivax
LNQKQPTKGSNIQ

SEQ ID NO: 290 - protein, 8 aa, Plasmodium vivax
LRPKKKLK

SEQ ID NO: 291 - protein, 8 aa, Plasmodium vivax
LSAAPAGV

SEQ ID NO: 292 - protein, 13 aa, Plasmodium vivax
MKQKGFGGQTKPV

SEQ ID NO: 293 - protein, 9 aa, Plasmodium vivax
MYKKVYVID

SEQ ID NO: 294 - protein, 9 aa, Plasmodium vivax
MSCDTSASA

SEQ ID NO: 295 - protein, 11 aa, Plasmodium vivax
MVSGTTGSTAN

SEQ ID NO: 296 - protein, 9 aa, Plasmodium vivax
MYKKVYVID

SEQ ID NO: 297 - protein, 12 aa, Plasmodium vivax
NAKGKKPAKKVI

SEQ ID NO: 298 - protein, 13 aa, Plasmodium vivax
NAQLTKQKTKKVI

SEQ ID NO: 299 - protein, 9 aa, Plasmodium vivax
NCAQGHCSQ

SEQ ID NO: 300 - protein, 13 aa, Plasmodium vivax
NEGDPSKGEGAET

SEQ ID NO: 301 - protein, 11 aa, Plasmodium vivax
NEKKELKTEAL

SEQ ID NO: 302 - protein, 8 aa, Plasmodium vivax
NFDKYHPG

SEQ ID NO: 303 - protein, 9 aa, Plasmodium vivax
NFDVAAERF

SEQ ID NO: 304 - protein, 10 aa, Plasmodium vivax
NFSKNIKKKK

SEQ ID NO: 305 - protein, 8 aa, Plasmodium vivax
NIPPKAFG

SEQ ID NO: 306 - protein, 11 aa, Plasmodium vivax
NKALLPTAGDD

SEQ ID NO: 307 - protein, 9 aa, Plasmodium vivax
NKEKLNHAV

SEQ ID NO: 308 - protein, 10 aa, Plasmodium vivax
NKEKLNHAVF

SEQ ID NO: 309 - protein, 14 aa, Plasmodium vivax
NKKGTPNTKKEPLL

SEQ ID NO: 310 - protein, 10 aa, Plasmodium vivax
NKKVYKLDKE

SEQ ID NO: 311 - protein, 11 aa, Plasmodium vivax
NKNSLTNFAVR

SEQ ID NO: 312 - protein, 15 aa, Plasmodium vivax
NKVRPIRTPGGKLTI

SEQ ID NO: 313 - protein, 13 aa, Plasmodium vivax
NLKGAKAEEGKKD

SEQ ID NO: 314 - protein, 11 aa, Plasmodium vivax
NNDFQKLESYD

SEQ ID NO: 315 - protein, 9 aa, Plasmodium vivax
NPFNRYPAY

SEQ ID NO: 316 - protein, 12 aa, Plasmodium vivax
NQKQPTKGSNIQ

SEQ ID NO: 317 - protein, 10 aa, Plasmodium vivax
NQLRPKKKLK

SEQ ID NO: 318 - protein, 9 aa, Plasmodium vivax
NSLTNFAVR

SEQ ID NO: 319 - protein, 14 aa, Plasmodium vivax
NSVKSNKKVKKMIK

SEQ ID NO: 320 - protein, 10 aa, Plasmodium vivax
NTIAFVATEK

SEQ ID NO: 321 - protein, 8 aa, Plasmodium vivax
NVCYRVCC

SEQ ID NO: 322 - protein, 10 aa, Plasmodium vivax
NVKGNPKAAA

SEQ ID NO: 323 - protein, 10 aa, Plasmodium vivax
PGRGAPLAKI

SEQ ID NO: 324 - protein, 8 aa, Plasmodium vivax
PKFFKNQR

SEQ ID NO: 325 - protein, 9 aa, Plasmodium vivax
PKFFKNQRY

SEQ ID NO: 326 - protein, 15 aa, Plasmodium vivax
PKIEPPKKKFIPSVL

SEQ ID NO: 327 - protein, 10 aa, Plasmodium vivax
PLPDRNDVPL

SEQ ID NO: 328 - protein, 9 aa, Plasmodium vivax
PLSNKKTVK

SEQ ID NO: 329 - protein, 8 aa, Plasmodium vivax
PPKDVVPS

SEQ ID NO: 330 - protein, 14 aa, Plasmodium vivax
PPKERKTKEQIAAA

SEQ ID NO: 331 - protein, 12 aa, Plasmodium vivax
PPSGGSPNRSPP

SEQ ID NO: 332 - protein, 13 aa, Plasmodium vivax
PQKEDAKGGKKKK

SEQ ID NO: 333 - protein, 13 aa, Plasmodium vivax
PRNPNYRDQQYPD

SEQ ID NO: 334 - protein, 9 aa, Plasmodium vivax
QFTKQRSNI

SEQ ID NO: 335 - protein, 11 aa, Plasmodium vivax
QKKPAAPETSA

SEQ ID NO: 336 - protein, 11 aa, Plasmodium vivax
QKQPTKGSNIQ

SEQ ID NO: 337 - protein, 10 aa, Plasmodium vivax
QRSALVNNPL

SEQ ID NO: 338 - protein, 10 aa, Plasmodium vivax
RAAPEEHPVL

SEQ ID NO: 339 - protein, 9 aa, Plasmodium vivax
RGSAEDDLK

SEQ ID NO: 340 - protein, 14 aa, Plasmodium vivax
RAGKVKNQTPKVPK

SEQ ID NO: 341 - protein, 15 aa, Plasmodium vivax
RAISKNGKNRFIKPK

SEQ ID NO: 342 - protein, 15 aa, Plasmodium vivax
RGETDVETRQNNILL

SEQ ID NO: 343 - protein, 12 aa, Plasmodium vivax
RKAHKNGIKKPK

SEQ ID NO: 344 - protein, 9 aa, Plasmodium vivax
RKKGPNSKL

SEQ ID NO: 345 - protein, 14 aa, Plasmodium vivax
RKKPATPKKQATPK

SEQ ID NO: 346 - protein, 15 aa, Plasmodium vivax
RKKPATPKKQATPKK

SEQ ID NO: 347 - protein, 9 aa, Plasmodium vivax
RKYKIILAF

SEQ ID NO: 348 - protein, 10 aa, Plasmodium vivax
RLELTPKQKV

SEQ ID NO: 349 - protein, 10 aa, Plasmodium vivax
RLTGGKKKIH

SEQ ID NO: 350 - protein, 11 aa, Plasmodium vivax
RLTGGKKKIHK

SEQ ID NO: 351 - protein, 13 aa, Plasmodium vivax
RLTGGKKKIHKKK

SEQ ID NO: 352 - protein, 11 aa, Plasmodium vivax
RNKKIYRIGLK

SEQ ID NO: 353 - protein, 13 aa, Plasmodium vivax
RNLKKSIKKKPKS

SEQ ID NO: 354 - protein, 14 aa, Plasmodium vivax
RNLKKSIKKKPKSK

SEQ ID NO: 355 - protein, 13 aa, Plasmodium vivax
RPPSNTKLGSKQV

SEQ ID NO: 356 - protein, 14 aa, Plasmodium vivax
RSSGLTNSRQQKMK

SEQ ID NO: 357 - protein, 8 aa, Plasmodium vivax
RSYSFNSM

SEQ ID NO: 358 - protein, 9 aa, Plasmodium vivax
RTPGGKLTI

SEQ ID NO: 359 - protein, 11 aa, Plasmodium vivax
RTVGVSKKKGA

SEQ ID NO: 360 - protein, 15 aa, Plasmodium vivax
SAGIKKPHRYRPGTV

SEQ ID NO: 361 - protein, 14 aa, Plasmodium vivax
SDGTGRKKGPNSKL

SEQ ID NO: 362 - protein, 8 aa, Plasmodium vivax
SDIIKTNE

SEQ ID NO: 363 - protein, 13 aa, Plasmodium vivax
SFFNSKKIKKGSK

SEQ ID NO: 364 - protein, 14 aa, Plasmodium vivax
SFFNSKKIKKGSKS

SEQ ID NO: 365 - protein, 11 aa, Plasmodium vivax
SGFLLHPSVTF

SEQ ID NO: 366 - protein, 11 aa, Plasmodium vivax
SGGVLPNIHNV

SEQ ID NO: 367 - protein, 13 aa, Plasmodium vivax
SGKSTTTGHIIYK

SEQ ID NO: 368 - protein, 10 aa, Plasmodium vivax
SKDGKNEAAL

SEQ ID NO: 369 - protein, 11 aa, Plasmodium vivax
SKGPDTPIITN

SEQ ID NO: 370 - protein, 12 aa, Plasmodium vivax
SKNGKNRFIKPK

SEQ ID NO: 371 - protein, 14 aa, Plasmodium vivax
SKNGKNRFIKPKIQ

SEQ ID NO: 372 - protein, 14 aa, Plasmodium vivax
SKQNFAKNKKKAAN

SEQ ID NO: 373 - protein, 10 aa, Plasmodium vivax
SLALQKKKAA

SEQ ID NO: 374 - protein, 14 aa, Plasmodium vivax
SLGKQVGGKNQQVK

SEQ ID NO: 375 - protein, 15 aa, Plasmodium vivax
SLLALFKEKKEKPRS

SEQ ID NO: 376 - protein, 11 aa, Plasmodium vivax
SLTTPAAVAAK

SEQ ID NO: 377 - protein, 9 aa, Plasmodium vivax
SLVKQRSNI

SEQ ID NO: 378 - protein, 13 aa, Plasmodium vivax
SMKNKKDKTPPSK

SEQ ID NO: 379 - protein, 8 aa, Plasmodium vivax
SMCETTET

SEQ ID NO: 380 - protein, 15 aa, Plasmodium vivax
SNDDGNGKKFNKKPF

SEQ ID NO: 381 - protein, 10 aa, Plasmodium vivax
SNKKVKKMIK

SEQ ID NO: 382 - protein, 11 aa, Plasmodium vivax
SNMESDDAGDG

SEQ ID NO: 383 - protein, 9 aa, Plasmodium vivax
SQKLYTKVA

SEQ ID NO: 384 - protein, 11 aa, Plasmodium vivax
SRKGLDPKFFK

SEQ ID NO: 385 - protein, 9 aa, Plasmodium vivax
SSHAKGIVV

SEQ ID NO: 386 - protein, 12 aa, Plasmodium vivax
SSHAKGIVVEKV

SEQ ID NO: 387 - protein, 10 aa, Plasmodium vivax
STTTGHIIYK

SEQ ID NO: 388 - protein, 10 aa, Plasmodium vivax
STVITDQYVS

SEQ ID NO: 389 - protein, 14 aa, Plasmodium vivax
SVINAKAKLQKTEE

SEQ ID NO: 390 - protein, 13 aa, Plasmodium vivax
SVKSNKKVKKMIK

SEQ ID NO: 391 - protein, 12 aa, Plasmodium vivax
SYLFKKIKKKVF

SEQ ID NO: 392 - protein, 15 aa, Plasmodium vivax
TDEDAGKKKKVKKSL

SEQ ID NO: 393 - protein, 15 aa, Plasmodium vivax
TDEDAGKKKKVKKSL

SEQ ID NO: 394 - protein, 11 aa, Plasmodium vivax
TEGSTPKPKQR

SEQ ID NO: 395 - protein, 9 aa, Plasmodium vivax
TEYPPLGRF

SEQ ID NO: 396 - protein, 10 aa, Plasmodium vivax
TEYPPLGRFA

SEQ ID NO: 397 - protein, 10 aa, Plasmodium vivax
TFLFNKKKKK

SEQ ID NO: 398 - protein, 12 aa, Plasmodium vivax
TGKYGTRYGSSL

SEQ ID NO: 399 - protein, 8 aa, Plasmodium vivax
TGLLRGAK

SEQ ID NO: 400 - protein, 14 aa, Plasmodium vivax
TGLLRGAKKTKLVG

SEQ ID NO: 401 - protein, 11 aa, Plasmodium vivax
TGRKKGPNSKL

SEQ ID NO: 402 - protein, 8 aa, Plasmodium vivax
TKILIVHV

SEQ ID NO: 403 - protein, 9 aa, Plasmodium vivax
TKLVGKTED

SEQ ID NO: 404 - protein, 10 aa, Plasmodium vivax
TKRNLKKSIK

SEQ ID NO: 405 - protein, 14 aa, Plasmodium vivax
TLESPDNAEIDMSS

SEQ ID NO: 406 - protein, 14 aa, Plasmodium vivax
TLESPDNAEIDMSS

SEQ ID NO: 407 - protein, 8 aa, Plasmodium vivax
TPGGKLTI

SEQ ID NO: 408 - protein, 9 aa, Plasmodium vivax
TPIEKLHPI

SEQ ID NO: 409 - protein, 10 aa, Plasmodium vivax
TPIITNKPFG

SEQ ID NO: 410 - protein, 11 aa, Plasmodium vivax
TPIITNKPFGK

SEQ ID NO: 411 - protein, 13 aa, Plasmodium vivax
TSNSAKAGLQFPV

SEQ ID NO: 412 - protein, 9 aa, Plasmodium vivax
TTKVKRVQT

SEQ ID NO: 413 - protein, 10 aa, Plasmodium vivax
TTKVKRVQTF

SEQ ID NO: 414 - protein, 13 aa, Plasmodium vivax
VAKKESKIIKKQK

SEQ ID NO: 415 - protein, 14 aa, Plasmodium vivax
VAKKESKIIKKQKK

SEQ ID NO: 416 - protein, 12 aa, Plasmodium vivax
VETEPDDIDYGK

SEQ ID NO: 417 - protein, 14 aa, Plasmodium vivax
VETEPDDIDYGKSD

SEQ ID NO: 418 - protein, 15 aa, Plasmodium vivax
VETEPDDIDYGKSDD

SEQ ID NO: 419 - protein, 13 aa, Plasmodium vivax
VFPYDNTLPKYKF

SEQ ID NO: 420 - protein, 11 aa, Plasmodium vivax
VGDSDIIKTNE

SEQ ID NO: 421 - protein, 8 aa, Plasmodium vivax
VGNILLGV

SEQ ID NO: 422 - protein, 15 aa, Plasmodium vivax
VITDVGDSDIIKTNE

SEQ ID NO: 423 - protein, 15 aa, Plasmodium vivax
VKEVIKRKNVIGIIP

SEQ ID NO: 424 - protein, 9 aa, Plasmodium vivax
VKYAKKLRD

SEQ ID NO: 425 - protein, 9 aa, Plasmodium vivax
VNVPKTRKT

SEQ ID NO: 426 - protein, 10 aa, Plasmodium vivax
VNVPKTRKTY

SEQ ID NO: 427 - protein, 10 aa, Plasmodium vivax
VNVPKTRKTY

SEQ ID NO: 428 - protein, 8 aa, Plasmodium vivax
VPNGGMYL

SEQ ID NO: 429 - protein, 15 aa, Plasmodium vivax
VRVADNSLKTNIHQY

SEQ ID NO: 430 - protein, 11 aa, Plasmodium vivax
VSEVTTVEKDE

SEQ ID NO: 431 - protein, 12 aa, Plasmodium vivax
VSKRKKLTGRAK

SEQ ID NO: 432 - protein, 13 aa, Plasmodium vivax
VSKRKKLTGRAKK

SEQ ID NO: 433 - protein, 8 aa, Plasmodium vivax
VVAPPERK

SEQ ID NO: 434 - protein, 12 aa, Plasmodium vivax
VVVVKGQPRKLK

SEQ ID NO: 435 - protein, 10 aa, Plasmodium vivax
VYLIKILMIK

SEQ ID NO: 436 - protein, 8 aa, Plasmodium vivax
WGKYQKMK

SEQ ID NO: 437 - protein, 11 aa, Plasmodium vivax
WNYKAIRKIAK

SEQ ID NO: 438 - protein, 8 aa, Plasmodium vivax
YAANWGGT

SEQ ID NO: 439 - protein, 9 aa, Plasmodium vivax
YESIEVSKI

SEQ ID NO: 440 - protein, 10 aa, Plasmodium vivax
YESIEVSKID

SEQ ID NO: 441 - protein, 9 aa, Plasmodium vivax
YFDLSRASF

SEQ ID NO: 442 - protein, 10 aa, Plasmodium vivax
YFDLSRASFS

SEQ ID NO: 443 - protein, 10 aa, Plasmodium vivax
YGPLKKDLKA

SEQ ID NO: 444 - protein, 12 aa, Plasmodium vivax
YGRIFKKKITKK

SEQ ID NO: 445 - protein, 13 aa, Plasmodium vivax
YGRIFKKKITKKN

SEQ ID NO: 446 - protein, 11 aa, Plasmodium vivax
YINKVYLFVYN

SEQ ID NO: 447 - protein, 10 aa, Plasmodium vivax
YKILIKDKLK

SEQ ID NO: 448 - protein, 8 aa, Plasmodium vivax
YLNDLCRN

SEQ ID NO: 449 - protein, 15 aa, Plasmodium vivax
YRGDVVPKDVNAAVA

SEQ ID NO: 450 - protein, 10 aa, Plasmodium vivax
YRGVVTEEGA

SEQ ID NO: 451 - protein, 8 aa, Plasmodium vivax
YRVKGKKK

SEQ ID NO: 452 - protein, 9 aa, Plasmodium vivax
YYDNGDNHN

SEQ ID NO: 453 - protein, 14 aa, Plasmodium vivax
YYRVKGKKKILIPV

SEQ ID NO: 454 - protein, 12 aa, Plasmodium vivax
TLSKKVVNRAPK

SEQ ID NO: 455 - protein, 14 aa, Plasmodium vivax
TTKVKRVQTFGKKK

SEQ ID NO: 456 - protein, 11 aa, Plasmodium vivax
KDCFSSSCGKT

SEQ ID NO: 457 - protein, 9 aa, Plasmodium vivax
HAVFIDKAL

SEQ ID NO: 458 - protein, 15 aa, Plasmodium vivax
PPKERKTKEQIAAAA

SEQ ID NO: 459 - protein, 15 aa, Plasmodium vivax
NISVLEPKTETIEAL

SEQ ID NO: 460 - protein, 8 aa, Plasmodium vivax
KERNTKPF

SEQ ID NO: 461 - protein, 12 aa, Plasmodium vivax
VRVADNSLKTNI

SEQ ID NO: 462 - protein, 13 aa, Plasmodium vivax
KEKKQLYKGKVKK

SEQ ID NO: 463 - protein, 8 aa, Plasmodium vivax
KKNAKNVK

SEQ ID NO: 464 - protein, 14 aa, Plasmodium vivax
EAKNKSRMAGKEKD

SEQ ID NO: 465 - protein, 8 aa, Plasmodium vivax
KGKKPAKK

SEQ ID NO: 466 - protein, 10 aa, Plasmodium vivax
GFNSGHVVTK

SEQ ID NO: 467 - protein, 13 aa, Plasmodium vivax
KKSKTKKNTIITK

SEQ ID NO: 468 - protein, 13 aa, Plasmodium vivax
EMGADKKKKGAVY

SEQ ID NO: 469 - protein, 13 aa, Plasmodium vivax
KKKITKKNYILPK

SEQ ID NO: 470 - protein, 13 aa, Plasmodium vivax
GGKSKGKRSGTRY

SEQ ID NO: 471 - protein, 14 aa, Plasmodium vivax
CASCGYPSAKKRRF

SEQ ID NO: 472 - protein, 14 aa, Plasmodium vivax
KEPLLGGLNQKQPT

SEQ ID NO: 473 - protein, 8 aa, Plasmodium vivax
AGADSKSL

SEQ ID NO: 474 - protein, 14 aa, Plasmodium vivax
VSLEPKKPMVVETF

SEQ ID NO: 475 - protein, 118 aa, Plasmodium falciparum
MSKLMKGAIDNEKYRLRRIRIALTSKNLRAIEKVCSDIMKGAKEKNLNVSGPVRLPVKTLRITTRKSPCGEGTNTWDRFELRIYKRLIDLYSQCEVVTQMTSINIDPVVEVEVIITDS

SEQ ID NO: 476 - protein, 11 aa, Plasmodium falciparum
AAEEGAKAGAL

SEQ ID NO: 477 - protein, 11 aa, Plasmodium falciparum
DNNNYDDDEII

SEQ ID NO: 478 - protein, 13 aa, Plasmodium falciparum
EEYDESGPSIVHR

SEQ ID NO: 479 - protein, 10 aa, Plasmodium falciparum
GGATGAGLAL

SEQ ID NO: 480 - protein, 16 aa, Plasmodium falciparum
GKEKTHINLVVIGHVD

SEQ ID NO: 481 - protein, 10 aa, Plasmodium falciparum
HGNNMNTCLM

SEQ ID NO: 482 - protein, 9 aa, Plasmodium falciparum
KIYEKKILK

SEQ ID NO: 483 - protein, 8 aa, Plasmodium falciparum
KTATLGVI

SEQ ID NO: 484 - protein, 8 aa, Plasmodium falciparum
LEGKELPG

SEQ ID NO: 485 - protein, 16 aa, Plasmodium falciparum
LVITDVGDSDIIKTNE

SEQ ID NO: 486 - protein, 9 aa, Plasmodium falciparum
NEAEEFEDY

SEQ ID NO: 487 - protein, 9 aa, Plasmodium falciparum
PEEVAEELV

SEQ ID NO: 488 - protein, 8 aa, Plasmodium falciparum
PQNINEYF

SEQ ID NO: 489 - protein, 10 aa, Plasmodium falciparum
QGGGSPLLGT

SEQ ID NO: 490 - protein, 11 aa, Plasmodium falciparum
QGISDDSSIHH

SEQ ID NO: 491 - protein, 9 aa, Plasmodium falciparum
SLGSSILTK

SEQ ID NO: 492 - protein, 10 aa, Plasmodium falciparum
SLNDALIVSI

SEQ ID NO: 493 - protein, 8 aa, Plasmodium falciparum
VANKIGIL

SEQ ID NO: 494 - protein, 15 aa, Plasmodium falciparum
VITDVGDSDIIKTNE

SEQ ID NO: 495 - protein, 8 aa, Plasmodium falciparum
VLPELNGK